European Patent Application EP 4 524 246 A2, published March 19, 2025. Title: METHODS AND COMPOSITIONS FOR THE EXTRACTION AND AMPLIFICATION OF NUCLEIC ACID FROM A SAMPLE. Applicant: SEQUENOM, INC. The sequence listing filed with the application follows.

SEQUENCE LISTING (5 sequences)

SEQ ID NO: 1 - DNA, 20 bp, synthetic construct
  misc_feature 1..20: note = Description of artificial sequence: 5' adapter
  source 1..20: mol_type = other DNA
acacggcgcacgcctccacg

SEQ ID NO: 2 - DNA, 12 bp, synthetic construct
  misc_feature 1..12: note = Description of artificial sequence: 3' adapter
  source 1..12: mol_type = other DNA
cgtggaggcgtg

SEQ ID NO: 3 - DNA, 20 bp, synthetic construct
  misc_feature 1..20: note = Description of artificial sequence: 5' adapter
  source 1..20: mol_type = other DNA
acacggcgcacgcctccacg

SEQ ID NO: 4 - DNA, 12 bp, synthetic construct
  misc_feature 1..12: note = Description of artificial sequence: 3' adapter
  source 1..12: mol_type = other DNA
gtgcggaggtgc

SEQ ID NO: 5 - DNA, 13 bp, synthetic construct
  misc_feature 1..13: note = Description of artificial sequence: SSGA13dd3' 13 nucleobases with a dideoxy-nucleotide at its 3' position.
  source 1..13: mol_type = other DNA
  misc_difference 13: note = any dideoxy-nucleotide
cgtggaggcgtgn